European Patent Specification EP 4 038 197 B1, published January 29, 2025. Title: ASSAY METHODS AND KITS FOR DETECTING RARE SEQUENCE VARIANTS. Applicant: Rutgers Biomedical and Health Sciences (PHRI) Kramer, Fred R. Vargas-Gold, Diana R. The sequence listing filed with the application follows.

SEQUENCE LISTING (25 sequences)

SEQ ID NO: 1 - DNA, 89 bp, Artificial
  Synthetic
acctgccgtcaacacgtgcgcagtagaccatctctcttgaggatcttgaaggaaactgaacctctccaacgaatctcgaaaagtgctgt

SEQ ID NO: 2 - DNA, 51 bp, Artificial
  Synthetic
ccagggaccttaccttatacaccggatcctaactgaggtccaaccggagca

SEQ ID NO: 3 - DNA, 24 bp, Artificial
  Synthetic
ccagggaccttaccttatacaccg

SEQ ID NO: 4 - DNA, 46 bp, Artificial
  Synthetic
ccgcctgacctgccgtcaacacgtgcgcagtagaccatccaggcgg

SEQ ID NO: 5 - DNA, 55 bp, Artificial
  Synthetic
cgcctgctgggcatctgcctcacccaacacgtgcgcagtagaccacgctcatcat

SEQ ID NO: 6 - DNA, 41 bp, Artificial
  Synthetic
tttgtgttcccggacatagtccaatcttcggtggagctgca

SEQ ID NO: 7 - DNA, 23 bp, Artificial
  Synthetic
tttgtgttcccggacatagtcca

SEQ ID NO: 8 - DNA, 27 bp, Artificial
  Synthetic
tggtctcaacacgtgcgcagtagacca

SEQ ID NO: 9 - DNA, 55 bp, Artificial
  Synthetic
gccgcctgctgggcatctgcctcaaagaatcaacaagctacaactcgctcatcat

SEQ ID NO: 10 - DNA, 44 bp, Artificial
  Synthetic
ctgcctcacctccaccgtgcaagcactcgcagaaccttcggctc

SEQ ID NO: 11 - DNA, 21 bp, Artificial
  Synthetic
caccagttgagcaggtactgg

SEQ ID NO: 12 - DNA, 34 bp, Artificial
  Synthetic
ccgtggctggactatgtccgggaacacaccacgg

SEQ ID NO: 13 - DNA, 59 bp, Artificial
  Synthetic
ttgagcaggtactgggagccaatattgtctgtcctttacaagcacgagtgccaggaggg

SEQ ID NO: 14 - DNA, 30 bp, Artificial
  Synthetic
ccgtcgcagctcatgcccttcggccgacgg

SEQ ID NO: 15 - DNA, 22 bp, Artificial
  Synthetic
tcccggacatagtccaggaagg

SEQ ID NO: 16 - DNA, 88 bp, Artificial
  Synthetic
acctgccgtcaacacgtgcgcagtagaccatcggcctgctgaaaatgactgaatataaacacacagtctgagcccactctggagctga

SEQ ID NO: 17 - DNA, 52 bp, Artificial
  Synthetic
aaatgattctgaattagctgtatcgtcaagtacccagctactaatacgccat

SEQ ID NO: 18 - DNA, 45 bp, Artificial
  Synthetic
caacactggcgcagtagaccataaacttgtggtagttggagcgga

SEQ ID NO: 19 - DNA, 21 bp, Artificial
  Synthetic
aggcactcttgcctacgccat

SEQ ID NO: 20 - DNA, 27 bp, Artificial
  Synthetic
tggtctcaacactggcgcagtagacca

SEQ ID NO: 21 - DNA, 89 bp, Artificial
  Synthetic
acgtgccctcaatacgagcccccttcaccaactctcttgaggatcttgaaggaaactgaacctctccaacgaatctcgaaaagtgctgt

SEQ ID NO: 22 - DNA, 44 bp, Artificial
  Synthetic
cgcctgacgtgccctcaatacgagcccccttcaccaaccaggcg

SEQ ID NO: 23 - DNA, 51 bp, Artificial
  Synthetic
ccaaccgcgagaagatgacccaggcatagccagctaatgacccctcttctg

SEQ ID NO: 24 - DNA, 27 bp, Artificial
  Synthetic
cggctaagagaaccagtgagaaagggc

SEQ ID NO: 25 - DNA, 30 bp, Artificial
  Synthetic
ccgctccctccttcctggcctcccgagcgg